European Patent Specification EP 3 495 505 B1, published September 11, 2024. Title: QUANTITATIVE ASSESSMENT FOR CAP EFFICIENCY OF MESSENGER RNA. Applicant: Shire Human Genetic Therapies, Inc. Application PCT/US2014/027602. The sequence listing filed with the application follows.

SEQUENCE LISTING (8 sequences)

SEQ ID NO: 1 - RNA, 582 nt, Artificial Sequence
  chemically synthesized oligonucleotide
augggggugcacgaauguccugccuggcuguggcuucuccugucccugcugucgcucccucugggccucccaguccugggcgccccaccacgccucaucugugacagccgaguccuggagagguaccucuuggaggccaaggaggccgagaauaucacgacgggcugugcugaacacugcagcuugaaugagaauaucacugucccagacaccaaaguuaauuucuaugccuggaagaggauggaggucgggcagcaggccguagaagucuggcagggccuggcccugcugucggaagcuguccugcggggccaggcccuguuggucaacucuucccagccgugggagccccugcagcugcauguggauaaagccgucaguggccuucgcagccucaccacucugcuucgggcucugggagcccagaaggaagccaucuccccuccagaugcggccucagcugcuccacuccgaacaaucacugcugacacuuuccgcaaacucuuccgagucuacuccaauuuccuccggggaaagcugaagcuguacacaggggaggccugcaggacaggggacagauga

SEQ ID NO: 2 - RNA, 1652 nt, Artificial Sequence
  chemically synthesized oligonucleotide
auggaagaugccaaaaacauuaagaagggcccagcgccauucuacccacucgaagacgggaccgccggcgagcagcugcacaaagccaugaagcgcuacgcccuggugcccggcaccaucgccuuuaccgacgcacauaucgagguggacauuaccuacgccgaguacuucgagaugagcguucggcuggcagaagcuaugaagcgcuaugggcugaauacaaaccaucggaucguggugugcagcgagaauagcuugcaguucuucaugcccguguugggugcccuguucaucgguguggcuguggccccagcuaacgacaucuacaacgagcgcgagcugcugaacagcaugggcaucagccagcccaccgucguauucgugagcaagaaagggcugcaaaagauccucaacgugcaaaagaagcuaccgaucauacaaaagaucaucaucauggauagcaagaccgacuaccagggcuuccaaagcauguacaccuucgugacuucccauuugccacccggcuucaacgaguacgacuucgugcccgagagcuucgaccgggacaaaaccaucgcccugaucaugaacaguaguggcaguaccggauugcccaagggcguagcccuaccgcaccgcaccgcuuguguccgauucagucaugcccgcgaccccaucuucggcaaccagaucauccccgacaccgcuauccucagcguggugccauuucaccacggcuucggcauguucaccacgcugggcuacuugaucugcggcuuucgggucgugcucauguaccgcuucgaggaggagcuauucuugcgcagcuugcaagacuauaagauucaaucugcccugcuggugcccacacuauuuagcuucuucgcuaagagcacucucaucgacaaguacgaccuaagcaacuugcacgagaucgccagcggcggggcgccgcucagcaaggagguaggugaggccguggccaaacgcuuccaccuaccaggcauccgccagggcuacggccugacagaaacaaccagcgccauucugaucacccccgaaggggacgacaagccuggcgcaguaggcaagguggugcccuucuucgaggcuaaggugguggacuuggacaccgguaagacacugggugugaaccagcgcggcgagcugugcguccguggccccaugaucaugagcggcuacguuaacaaccccgaggcuacaaacgcucucaucgacaaggacggcuggcugcacagcggcgacaucgccuacugggacgaggacgagcacuucuucaucguggaccggcugaagagccugaucaaauacaagggcuaccagguagccccagccgaacuggagagcauccugcugcaacaccccaacaucuucgacgccggggucgccggccugcccgacgacgaugccggcgagcugcccgccgcagucgucgugcuggaacacgguaaaaccaugaccgagaaggagaucguggacuauguggccagccagguuacaaccgccaagaagcugcgcggugguguuguguucguggacgaggugccuaaaggacugaccggcaaguuggacgcccgcaagauccgcgagauucucauuaaggccaagaagggcggcaagaucgccgugua

SEQ ID NO: 3 - RNA, 140 nt, Artificial Sequence
  chemically synthesized oligonucleotide
ggacagaucgccuggagacgccauccacgcuguuuugaccuccauagaagacaccgggaccgauccagccuccgcggccgggaacggugcauuggaacgcggauuccccgugccaagagugacucaccguccuugacacg

SEQ ID NO: 4 - RNA, 11 nt, Artificial Sequence
  chemically synthesized oligonucleotide
gggauccuacc

SEQ ID NO: 5 - RNA, 100 nt, Artificial Sequence
  chemically synthesized oligonucleotide
cggguggcaucccugugaccccuccccagugccucuccuggcccuggaaguugccacuccagugcccaccagccuuguccuaauaaaauuaaguugcauc

SEQ ID NO: 6 - RNA, 8 nt, Artificial Sequence
  chemically synthesized oligonucleotide
uuugaauu

SEQ ID NO: 7 - RNA, 1290 nt, Artificial Sequence
  chemically synthesized oligonucleotide
augcagcugaggaacccagaacuacaucugggcugcgcgcuugcgcuucgcuuccuggcccucguuuccugggacaucccuggggcuagagcacuggacaauggauuggcaaggacgccuaccaugggcuggcugcacugggagcgcuucaugugcaaccuugacugccaggaagagccagauuccugcaucagugagaagcucuucauggagauggcagagcucauggucucagaaggcuggaaggaugcagguuaugaguaccucugcauugaugacuguuggauggcuccccaaagagauucagaaggcagacuucaggcagacccucagcgcuuuccucaugggauucgccagcuagcuaauuauguucacagcaaaggacugaagcuagggauuuaugcagauguuggaaauaaaaccugcgcaggcuucccugggaguuuuggauacuacgacauugaugcccagaccuuugcugacuggggaguagaucugcuaaaauuugaugguuguuacugugacaguuuggaaaauuuggcagaugguuauaagcacauguccuuggcccugaauaggacuggcagaagcauuguguacuccugugaguggccucuuuauauguggcccuuucaaaagcccaauuauacagaaauccgacaguacugcaaucacuggcgaaauuuugcugacauugaugauuccuggaaaaguauaaagaguaucuuggacuggacaucuuuuaaccaggagagaauuguugauguugcuggaccaggggguuggaaugacccagauauguuagugauuggcaacuuuggccucagcuggaaucagcaaguaacucagauggcccucugggcuaucauggcugcuccuuuauucaugucuaaugaccuccgacacaucagcccucaagccaaagcucuccuucaggauaaggacguaauugccaucaaucaggaccccuugggcaagcaaggguaccagcuuagacagggagacaacuuugaagugugggaacgaccucucucaggcuuagccugggcuguagcuaugauaaaccggcaggagauugguggaccucgcucuuauaccaucgcaguugcuucccuggguaaaggaguggccuguaauccugccugcuucaucacacagcuccucccugugaaaaggaagcuaggguucuaugaauggacuucaagguuaagaagucacauaaaucccacaggcacuguuuugcuucagcuagaaaauacaaugcagaugucauuaaaagacuuacuuuaa

SEQ ID NO: 8 - RNA, 1510 nt, Artificial Sequence
  chemically synthesized oligonucleotide
augcagcugaggaacccagagcuccaucucggaugugcacuggcacuuagauuucucgcgcuugugucgugggacauccccggagccagggcgcuggauaaugggcucgcccggacucccacaauggguuggcugcacugggagcgcuuuaugugcaaucuggacugccaggaagagcccgauagcuguauuucggagaagcucuucauggaaauggcggaguugaugguguccgaaggguggaaggaugcgggauaugaguaucuguguaucgaugacugcuggauggcaccgcagcgagauucggaggggcgauugcaggccgacccucagcgcuucccucauggaauucggcagcuggccaacuacguacacucaaaaggacuuaaguuggggaucuacgcggacgucgguaauaagacaugcgcuggguucccggggagcuucggauacuaugauauugaugcccagaccuucgcggacuggggaguggacuugcuuaaguuugaugguuguuacugugacucauuggaaaacuuggcggauggguauaaacauauguccuuggccuugaaucggacagggcggucgaucgucuacagcugcgaauggccuuuguauauguggccguuccagaaacccaacuacaccgaaauucgccaguauugcaaucacuggagaaacuucgccgauaucgacgauucguggaaaucaaucaaguccauccucgacuggacguccuucaaccaagagagaaucguagauguggccggaccgggaggauggaacgacccugauaugcuuguaauuggcaacuuuggacucucguggaaccagcaaguaacgcaaauggcacucugggcuaucauggcugcgccccuguucaugucaaacgaccucaggcacaucucgccgcaggcgaaagccuugcuucaagauaaggacgucaucgcgauuaaucaggacccgcuggggaagcagggcuaucagcuuagacagggcgacaauuuugaggucugggagcgaccccugagcggacucgcaugggcgguggcaaugaucaauaggcaggaaauuggugggccgaggucguacacuaucgccgucgcgucguugggaaaggguguggcguguaauccagcgugcuuuaucacccaacugcugcccgucaagcgcaaacuggguuuuuacgaauggacgagcagacuucgcucacacauuaacccaacggguacgguguugcuccagcucgagaauacaaugcaaaugucacuuaaagauuugcucugacggguggcaucccugugaccccuccccagugccucuccuggcccuggaaguugccacuccagugcccaccagccuuguccuaauaaaauuaaguugcaucaaaaaaaaaaaaaaaaaaaaaaaaaaaaaaaaaaaaaaaaaaaaaaaaaaaaaaaaaaaaaaaaaaaaaaaaaaaaaaaaaaaaaaaaaaaaaaaaaaaaaaaaaaaaaaaaaaaaaaaa